European Patent Application EP 4 379 045 A1, published June 5, 2024. Title: Method for producing highly proliferating cells, highly proliferating cells and use thereof. Applicant: Tokyo Medical University. Application JP. The sequence listing filed with the application follows.

SEQUENCE LISTING (28 sequences)

SEQ ID NO: 1 - DNA, 22 bp, synthetic construct
  misc_feature 1..22: note = forward primer for Notch1
  source 1..22: mol_type = other DNA
cacaaggtgtcttccagatcct

SEQ ID NO: 2 - DNA, 20 bp, synthetic construct
  misc_feature 1..20: note = reverse primer for Notch1
  source 1..20: mol_type = other DNA
ggcatccacattgttcacgg

SEQ ID NO: 3 - DNA, 20 bp, synthetic construct
  misc_feature 1..20: note = forward primer for Nestin
  source 1..20: mol_type = other DNA
gcgttggaacagaggttgga

SEQ ID NO: 4 - DNA, 20 bp, synthetic construct
  misc_feature 1..20: note = reverse primer for Nestin
  source 1..20: mol_type = other DNA
gagcgatctggctctgtagg

SEQ ID NO: 5 - DNA, 19 bp, synthetic construct
  misc_feature 1..19: note = forward primer for SOX2
  source 1..19: mol_type = other DNA
catggacagttacgcgcac

SEQ ID NO: 6 - DNA, 22 bp, synthetic construct
  misc_feature 1..22: note = reverse primer for SOX2
  source 1..22: mol_type = other DNA
agctggtcatggagttgtactg

SEQ ID NO: 7 - DNA, 22 bp, synthetic construct
  misc_feature 1..22: note = forward primer for S100B
  source 1..22: mol_type = other DNA
ggtgagacaaggaagaggatgt

SEQ ID NO: 8 - DNA, 21 bp, synthetic construct
  misc_feature 1..21: note = reverse primer for S100B
  source 1..21: mol_type = other DNA
gatgagctccttcagttcgga

SEQ ID NO: 9 - DNA, 22 bp, synthetic construct
  misc_feature 1..22: note = forward primer for NG2
  source 1..22: mol_type = other DNA
tgctgttctcacacagaggaac

SEQ ID NO: 10 - DNA, 20 bp, synthetic construct
  misc_feature 1..20: note = reverse primer for NG2
  source 1..20: mol_type = other DNA
ttcagcgagaggagcacttg

SEQ ID NO: 11 - DNA, 20 bp, synthetic construct
  misc_feature 1..20: note = forward primer for GFAP
  source 1..20: mol_type = other DNA
cttgcaggagtaccaggacc

SEQ ID NO: 12 - DNA, 20 bp, synthetic construct
  misc_feature 1..20: note = reverse primer for GFAP
  source 1..20: mol_type = other DNA
ttgaggtggccttctgacac

SEQ ID NO: 13 - DNA, 25 bp, synthetic construct
  misc_feature 1..25: note = forward primer for ACTB
  source 1..25: mol_type = other DNA
tgaaggtcggagtcaacgatttggt

SEQ ID NO: 14 - DNA, 20 bp, synthetic construct
  misc_feature 1..20: note = reverse primer for ACTB
  source 1..20: mol_type = other DNA
gaagatggtgatgggatttc

SEQ ID NO: 15 - DNA, 19 bp, synthetic construct
  misc_feature 1..19: note = forward primer for GAPDH
  source 1..19: mol_type = other DNA
attgccgacaggatgcaga

SEQ ID NO: 16 - DNA, 21 bp, synthetic construct
  misc_feature 1..21: note = reverse primer for GAPDH
  source 1..21: mol_type = other DNA
gagtacttgcgctcaggagga

SEQ ID NO: 17 - DNA, 20 bp, synthetic construct
  source 1..20: mol_type = other DNA
  misc_feature 1..20: note = forward primer for SLC1A2
gccggatagtgctgaagagg

SEQ ID NO: 18 - DNA, 21 bp, synthetic construct
  source 1..21: mol_type = other DNA
  misc_feature 1..21: note = reverse primer for SLC1A2
ggcatattgttggcaccttcc

SEQ ID NO: 19 - DNA, 18 bp, synthetic construct
  source 1..18: mol_type = other DNA
  misc_feature 1..18: note = forward primer for SLC1A3
tgacatctgtcggcctgc

SEQ ID NO: 20 - DNA, 18 bp, synthetic construct
  source 1..18: mol_type = other DNA
  misc_feature 1..18: note = reverse primer for SLC1A3
ggaggcgatccaggaacc

SEQ ID NO: 21 - DNA, 20 bp, synthetic construct
  source 1..20: mol_type = other DNA
  misc_feature 1..20: note = forward primer for OLIG2
atagatcgacgcgacaccag

SEQ ID NO: 22 - DNA, 20 bp, synthetic construct
  source 1..20: mol_type = other DNA
  misc_feature 1..20: note = reverse primer for OLIG2
ctttcgcagggtcctccttc

SEQ ID NO: 23 - DNA, 20 bp, synthetic construct
  source 1..20: mol_type = other DNA
  misc_feature 1..20: note = reverse primer for PAX6
caagcaacaacagcagcaca

SEQ ID NO: 24 - DNA, 21 bp, synthetic construct
  source 1..21: mol_type = other DNA
  misc_feature 1..21: note = reverse primer for PAX6
cggatgtctgtccactctcac

SEQ ID NO: 25 - DNA, 20 bp, synthetic construct
  source 1..20: mol_type = other DNA
  misc_feature 1..20: note = forward primer for ALDH1L1
cgtgcggagagtggtagaag

SEQ ID NO: 26 - DNA, 20 bp, synthetic construct
  source 1..20: mol_type = other DNA
  misc_feature 1..20: note = reverse primer for ALDH1L1
aattccgtgtagagcggacc

SEQ ID NO: 27 - DNA, 20 bp, synthetic construct
  source 1..20: mol_type = other DNA
  misc_feature 1..20: note = forward primer for MSI1
aattccgtgtagagcggacc

SEQ ID NO: 28 - DNA, 20 bp, synthetic construct
  source 1..20: mol_type = other DNA
  misc_feature 1..20: note = reverse primer for MSI1
gcagtgagaggaatggctgt